European Patent Application EP 4 616 723 A1, published September 17, 2025. Title: Fermented grains having gluten degradation activity, method of manufacturing the same and food composition comprising the same. Applicant: NaturePureKorea. The sequence listing filed with the application follows.

SEQUENCE LISTING (1 sequence)

SEQ ID NO: 1 - DNA, 1501 bp, synthetic construct
  source 1..1501: mol_type = other DNA
ttttttttttttttttttttttctcagacgaacgctggcggcgtgcctaatacatgcaagtcgagcggacagatgggagcttgctccctgatgttagcggcggacgggtgagtaacacgtgggtaacctgcctgtaagactgggataactccgggaaaccggggctaataccggatgcttgtttgaaccgcatggttcaaacataaaaggtggcttcggctaccacttacagatggacccgcggcgcattagctagttggtgaggtaacggctcaccaaggcgacgatgcgtagccgacctgagagggtgatcggccacactgggactgagacacggcccagactcctacgggaggcagcagtagggaatcttccgcaatggacgaaagtctgacggagcaacgccgcgtgagtgatgaaggttttcggatcgtaaagctctgttgttagggaagaacaagtgccgttcaaatagggcggcaccttgacggtacctaaccagaaagccacggctaactacgtgccagcagccgcggtaatacgtaggtggcaagcgttgtccggaattattgggcgtaaagggctcgcaggcggtttcttaagtctgatgtgaaagcccccggctcaaccggggagggtcattggaaactggggaacttgagtgcagaagaggagagtggaattccacgtgtagcggtgaaatgcgtagagatgtggaggaacaccagtggcgaaggcgactctctggtctgtaactgacgctgaggagcgaaagcgtggggagcgaacaggattagataccctggtagtccacgccgtaaacgatgagtgctaagtgttagggggtttccgccccttagtgctgcagctaacgcattaagcactccgcctggggagtacggtcgcaagactgaaactcaaaggaattgacgggggcccgcacaagcggtggagcatgtggtttaattcgaagcaacgcgaagaaccttaccaggtcttgacatcctctgacaatcctagagataggacgtccccttcgggggcagagtgacaggtggtgcatggttgtcgtcagctcgtgtcgtgagatgttgggttaagtcccgcaacgagcgcaacccttgatcttagttgccagcattcagttgggcactctaaggtgactgccggtgacaaaccggaggaaggtggggatgacgtcaaatcatcatgccccttatgacctgggctacacacgtgctacaatgggcagaacaaagggcagcgaaaccgcgaggttaagccaatcccacaaatctgttctcagttcggatcgcagtctgcaactcgactgcgtgaagctggaatcgctagtaatcgcggatcagcatgccgcggtgaatacgttcccgggccttgtacacaccgcccgtcacaccacgagagtttgtaacacccgaagtcggtgaggtaacctttttggagccagccgccgaaggtgggacagatgattggggtgaag